European Patent Specification EP 3 658 571 B1, published September 3, 2025. Title: OTOPETRIN PROTON CHANNELS AS TARGETS FOR PHARMACEUTICAL DISCOVERY. Applicant: UNIVERSITY OF SOUTHERN CALIFORNIA Liman, Emily Tu, Yu-Hsiang. Application To Be Assigned. The sequence listing filed with the application follows.

SEQUENCE LISTING (9 sequences)

SEQ ID NO: 1 - protein, 612 aa, Homo sapiens
MLEGLGSPASPRAAASASVAGSSGPAACSPPSSSAPRSPESPAPRRGGVRASVPQKLAEMLSSQYGLIVFVAGLLLLLAWAVHAAGVSKSDLLCFLTALMLLQLLWMLWYVGRSSAHRRLFRLKDTHAGAGWLRGSITLFAVITVILGCLKIGYFIGFSECLSATEGVFPVTHSVHTLLQVYFLWGHAKDIIQSFKTLERFGVIHSVFTNLLLWANGVLNESKHQLNEHKERLITLGFGNITTVLDDHTPQCNCTPPTLCTAISHGIYYLYPFNIEYQILASTMLYVLWKNIGRKVDSHQHQKMQFKSDGVMVGAVLGLTVLAATIAVVVVYLIHIGRSKTKSESALIMFYLYAITLLMLMGAAGLAGIRIYRIDEKSLDESKNPARKLDSDLLVGTASGSWLISWGSILAILCAEGHPRYTWYNLPYSILAIVEKYIQNLFIFESIHREPEKLSEDIQTLRVVTVCNGNTMPLASSCPKSGGVARDVAPQGKDMPPAANGNVCMRESHDKEEEKQEESSWGGSPSPVRLPRFLQGNAKRKVLRNIAAFLFLCNISLWIPPAFGCRPEYDNGLEEIVFGFEPWIIVVNLAMPFSIFYRMHAAASLFEVYCKI

SEQ ID NO: 2 - protein, 562 aa, Homo sapiens
MSEELAQGPKESPPAPRAGPREVWKKGGRLLSVLLAVNVLLLACTLISGGAFNKVAVYDTDVFALLTAMMLLATLWILFYLLRTVRCPCAVPYRDAHAGPIWLRGGLVLFGICTLIMDVFKTGYYSSFFECQSAIKILHPLIQAVFVIIQTYFLWVSAKDCVHVHLDLTWCGLMFTLTTNLAIWMAAVVDESVHQSHSYSSSHSNASHARLISDQHADNPVGGDSCLCSTAVCQIFQQGYFYLYPFNIEYSLFASTMLYVMWKNVGRFLASTPGHSHTPTPVSLFRETFFAGPVLGLLLFVVGLAVFIIYEVQVSGDGSRTRQALVIYYSFNIVCLGLTTLVSLSGSIIYRFDRRAMDHHKNPTRTLDVALLMGAALGQYAISYYSIVAVVAGTPQDLLAGLNLTHALLMIAQHTFQNMFIIESLHRGPPGAEPHSTHPKEPCQDLTFTNLDALHTLSACPPNPGLVSPSPSDQREAVAIVSTPRSQWRRQCLKDISLFLLLCNVILWIMPAFGARPHFSNTVEVDFYGYSLWAVIVNICLPFGIFYRMHAVSSLLEVYVLS

SEQ ID NO: 3 - protein, 596 aa, Homo sapiens
MGRGARAAAAQSRWGRASRASVSPGRTIRSAPAVGEAQETEAAPEKENRVDVGAEERAAATRPRQKSWLVRHFSLLLRRDRQAQKAGQLFSGLLALNVVFLGGAFICSMIFNKVAVTLGDVWILLATLKVLSLLWLLYYVASTTRRPHAVLYQDPHAGPLWVRGSLVLFGSCTFCLNIFRVGYDVSHIRCKSQLDLVFSVIEMVFIGVQTWVLWKHCKDCVRVQTNFTRCGLMLTLATNLLLWVLAVTNDSMHREIEAELGILMEKSTGNETNTCLCLNATACEAFRRGFLMLYPFSTEYCLICCAVLFVMWKNVGRHVAPHMGAHPATAPFHLHGAIFGPLLGLLVLLAGVCVFVLFQIEASGPAIACQYFTLYYAFYVAVLPTMSLACLAGTAIHGLEERELDTVKNPTRSLDVVLLMGAALGQMGIAYFSIVAIVAKRPHELLNRLILAYSLLLILQHIAQNLFIIEGLHRRPLWETVPEGLAGKQEAEPPRRGSLLELGQGLQRASLAYIHSYSHLNWKRRALKEISLFLILCNITLWMMPAFGIHPEFENGLEKDFYGYQIWFAIVNFGLPLGVFYRMHSVGGLVEVYLGA

SEQ ID NO: 4 - protein, 600 aa, Mus musculus
MPGGPGAPSSPAASSGSSRAAPSGIAACPLSPPPLARGSPQASGPRRGASVPQKLAETLSSQYGLNVFVAGLLFLLAWAVHATGVGKSDLLCVLTALMLLQLLWMLWYVGRSYMQRRLIRPKDTHAGARWLRGSITLFAFITVVLGCLKVAYFIGFSECLSATEGVFPVTHAVHTLLQVYFLWGHAKDIIMSFKTLERFGVIHSVFTNLLLWANSVLNESKHQLNEHKERLITLGFGNITIVLDDHTPQCNCTPPALCSALSHGIYYLYPFNIEYQILASTMLYVLWKNIGRRVDSSQHQKMQCRFDGVLVGSVLGLTVLAATIAVVVVYMIHIGRSKSKSESALIMFYLYAITVLLLMGAAGLVGSWIYRVDEKSLDESKNPARKLDVDLLVATASGSWLLSWGSILAIACAETRPPYTWYNLPYSVLVIVEKYVQNIFIIESVHLEPEGVPEDVRTLRVVTVCSSEAAALAASTLGSQGMAQDGSPAVNGNLCLQQRCGKEDQESGWEGATGTTRCLDFLQGGMKRRLLRNITAFLFLCNISLWIPPAFGCRPEYDNGLEEIVFGFEPWIIVVNLAMPFSIFYRMHAAAALFEVYCKI

SEQ ID NO: 5 - protein, 563 aa, Mus musculus
MSEELVPHPNESLPGPRASPREVWKKGGRLLSVLLAVNVLLLACTLISGGAFNKVAVYDTDVFALLTTMMLLAALWIVFYLLRTARCPDAVPYRDAHAGPIWLRGGLVLFGICTLVMDVFKTGYYSSFFECQSAIKILHPIIQAVFVIVQTYFLWISAKDCIHTHLDLTRCGLMFTLATNLAIWMAAVVDESVHQAHSYSGSHGNTSHTRLNPDSKRAGGAAEEDPCLCSTAICQIFQQGYFYLYPFNIEYSLFASTMLYVMWKNVGRLLASTHGHGHTPSRVSLFRETFFAGPVLGLLLFVVGLAVFILYEVQVSGERGHTRQALVIYYSFNIVCLGLMTLVSLSGSVIYRFDRRAMDHHKNPTRTLDVALLMGAALGQYAISYYSIVAVVVGSPRDLQGALNLSHALLMIAQHTFQNVFIIESLHRGPPGAEPREMPPKEPCQGITFANLDAIRTLPSCPPTPRLVIPNLESPQEAVAIISAPRCHWRRRCLKDISLFLLLCNVILWIMPAFGARPHFSNTVEVDFYGYSLWAAIVNICLPFGIFYRMHAVSSLLEVYVLS

SEQ ID NO: 6 - protein, 577 aa, Mus musculus
MASQTSAPAEPAPMPSPEAKTTEGASSYDQADMETKHAGSPCPPKQKSWLARHFSLLLRRDRQAQKAGQLFSGLLALNVVFLGGAFICSMIFNKVSVTLGDVWILLAALKVLSLLWLLYYTVGTTRKPHAVLYRDPHAGPIWVRGSLVLFGSCTVCLNIFRMGYDVSHIHCKSEVELIFPAIEIVFMIIQTWVLWRHCKDCVQVQTNFTRCGLMLTLATNLLMWVLAVTNDSMHREIEAELDALMEKFSGNGTNTCMCLNTTVCEVFRKGYLMLYPFSTEYCLICCAVLFVMWKNVSRSLAAHTGAHPNRSPFRLHGTIFGPLLGLLALVAGVCVFVLFQIEASGPDIARQYFTLYYAFYVAVLPTMSLACLAGTAIHGLEERELDTLKNPTRSLDVVLLMGAALGQMGIAYFSIVAIVATQPHELLNQLILAYSLLLILQHITQNLFIIEGLHRRPLWEPAVSGVMEKQDVELPRRGSLRELGQDLRRASRAYIHSFSHLNWKRRMLKEISLFLILCNITLWMMPAFGIHPEFENGLEKDFYGYRTWFTIVNFGLPLGVFYRMHSVGGLVEVYLGA

SEQ ID NO: 7 - protein, 977 aa, Drosophila
MQRCPYIHEMRERLLDQPRETLQLENMERANLLDNRQSASESNQLQGDGYHTSPAHQRTPLVPHDLGEDFNLDFDDDFPIDARRPKNANDIHPAVLTRPQQRTSLFIVTSLVYAILLIVVCIAYVISDVTTHRLPVLYYETFFTYLYGVSILFLLYVFCFLLQESSCCNGGNGGSKPKPQPKEKKSKKAKNADPADSKDAKGSKDSGKAAKGAAYQHTLAKFLEAPVDAEVAVTPKNVRKRKTTHSDLTHGSFFLRVGAIAFGLGAMIYIGLEFGSFFEIPFDSPCHHILIGVNPLLQMIFTFMQMYFIFMNARTRPPFQLNIHRFKVIARFGLMHVVATNICVWIRTLVKESLLEITIYHQKNEPEAGASSIAHSIRQHALRHAGTVLRTHAGPNSEFEVLDGEDILPKDVYKSDNVLSKLVRNTVDGISKSLGMGGDQALDSSTTSSSTTTTTRAPFTTPNYQWHSTTMARKLKKFITSATTAATTAAGSSSTASSTTTISPTISSTTIPSTTISSTTISSSTTFSPFSPSTTTTTTTTAAALNLETSGSESPFGGLQRILSSAAPPSLAPVDGFGSASAATPTSGSGAGSFVDSFLASTLSPASSTEGSASIMNNLFGQGPMENSFQTYTDLGHEEATGLVSFENLESLDNIYPAALSSNIGTLNSTACGRIDIMGTIVYDSAPYLYPFIIEYSLIGAVVLYVMWKHIGRYPGRMNDEDLEHRLEVMLSRRAVAMAQQARSGRVDCVGSSKGLFFGLLLLVGALICLILFFVLVRHQQFSLLAIYLADASHCILMAFAILAIIVGFIRVKNLKFRCEEQSNLNDILLRISAFGLFTYSVFSIIAGSLKVLESEPSLLVTTTGGVAVFQVILQLLFIADVSRRRVHLPEHDRSKPGRQIVTFLLICNVAMFAIYTFEAQKVFANPVSRYVQLEFYGFVPWSIIQRITLPLCIFHRFHSAVTLAEIWKTTYKARLE

SEQ ID NO: 8 - protein, 797 aa, Drosophila
MSLINLKSKDMYDEPINLWRTKQRVHYHHDVISKGNDSHRSSDACEYITISAPKKSGSFSRSPPSSLPTSVPGTPRHSVAATSNQVIRYARTSCDHCGHHSIPVMSPHPISPLAKSQTNLDLVEHGSQRQALLPLPTVGMHHEDSACTLQVSRRPSLLLQEILTQRPPLFGRRDGNGFLSPRTAKNGNLQGTASGSTATINFQSGATSARNGSTAFFDNGAKSFQAKQQKDKNRRTGNDAISSALSATYCKLLVLLGVCLPITEVISDQIPTYVYQGFYVYLYVGSILFVIFLYISAFRNRSLFNALKDYHEKNSNVHLKHKVTHFGSFYLRVGAIAFAIGTMVYSGLEFGQFFELNGHPGCRDVFVAITPICRMVLCIAQVQFIFLNTTYMDMARHKVTSRFGLMHMVATNLCEWLYVLVEETKHEIFHISQHEVDPAHDLVIHNSSMSRTDWAAVNESLHQHHHHHALNNTLVANVSSVIVNMTITPSPTPAAFSGCSRTTIMGALVQQLSPFLFPCTIEYSLICAVILFEMWKTVKSIPDIDKTRKNSVKPAAAKPAHHFSVDCSQSHKGLFFGILIIVMTIISMIMYFVLYTQPGYELVATQEVTLWETFMYFMCAAAVITGMILMRDLRYIKNTSDEHHSMDLDNLLLIVAQTGVYLYGMFSILGSYFAKWDTVPDRVEGIIAEVFGVVQTSLQTMFILHSSHRRCRGTNQVRRKPGREIITFLLVANIAIWFVNTLIKGRAVFRESHLEFFGVWGWTIITHISMPLAIFYRFHSTICLFEVWKITYKAKAH

SEQ ID NO: 9 - protein, 1576 aa, Drosophila
  misc_feature (1456)..(1456): Xaa can be any naturally occurring amino acid
MDSSPDLSLKLRRGSSDSRDNFYMDFAQGIDSDIEEVDNTANNQEAGEVPPPPLPTVSLAEEVLLLVAPPPPPPSLLGQPLPTLTETDDIPPTPTPPPQQKDDEGDDEDEREEPVPEQDQGAPAAPSPPGSPINSVLELELIPPPPLSPMDDAGLRTDDDGEGEETDDAEEVAAIPPPHEMLDIESNPDEEEEEEEQEQASQEDTPKEEDEEEDDDKSTPPPPLPPLPSNFSYVQGHNLGQVTPPLTKSPSNSPSPPVTPPPCPELNISRMVSPPAQHISQIPPLTPSDESEGEAESQPNSPPLRLDAEQPPPDMDQPEPEDQPPEPENEPEPEPEPEPEPEPVSGAREDYSRSLDNEDESTTITTPPSNGYSASSIIAPPPEHFAELDEDRGFIPPPPLEQEPEEEVEEEEEEEEEELTKETDEISVDRESLQDQGGDSISSPRPASILTGSISTSVGGGAGGSPKPESRGPSRSGSQRSQLRSGSQQGSIAESRGGSRIGSRTGSVASAQAAGVLSPQASLKSQTSIRSQGQAGVRSPAGSIKSGSQRMQSPQAGEGAPAMPSPPLMRSPPPELARQMHSPPRITTPPRVCSPPLVSSPPKLAESAAAAVGVAATVKEQIGSSSSTAEPLEPSKPEPLKPPIATVSYQDEQKPSPPPTAAAAPAVTTTAATTAVTSQPRSHFTSSHHHYHLPHQFQHPHHQNHHTHSVRVPTPTVPSSYAPPPPPDSGSSSSPVDRRRLFMAGVAPPIAAGAGSLMAMPAEPAVAISPGRVSARSGSQHHVTIDESSLPSHKGNIQETPGPSGLIIGGGDGDGDRDIGGGGGPDSSDPPSSPGGSSSQPALSGSQADGQLALMYHSHQLTNYPVLPAIKRTHRPSFVYPPMPRVKAGDALATLFSALYGKLLVVMGIAFPMAEVISTYIPPSFYEVYYLYLYIGSMIFLLFMYATLIWGRPKLPVPIASPSKSATKASGTDSMDESDTDSNSVHHRLPPPIPVRRPSLLSPLGRRDAHYGSFYLRMGAVAFGIGSMIYSGLEFGQYFELNPDTKCHNVLLALTPATRMAFIFIQMYFIFLNNEQIKVYRYKIIARFGLMHMIGTNLAVWLNVLIQETKHEILTFYNPENRTLRISHRIPGHSRGHAIIQHDPTAHLRVPRGLKGPYQIFECRRTNIIGTLVQDASPFLFPCTIEYSLICAAILYVMWRSISRPQTPTPQRPDMISSPMKRSPHHYSVDCARAHKGLFVGILILVLTIISLIIFFVLISRPEFVAMAVTEVTICELLIYGTATIATLVGMIQIRHLQYDAYRSFSLDDILLVGAQTGSFLYNIFTVIAGHFTLRSDDMLVPINALASIVQTACQTMFILDASRRQAVSPEHLRKKPGREIVTFMLVVNLAMWAISTLEKSRAESHPIQLNFYGLWAWTIITHVSMPLAIFYRFHSTVCLCEIWKRAYKLKPTYMXEFARSRIQSIAQQQQFCEDLKTNLSYCYCSTTLAGGELETVEEVDSGESNSAEDAGAGAGSGGSRGSGGGAGAAEAGEAGEEGQQGGDSSCGLKAPIRALSPQSLNTEKAFCPVYVINGE